European Patent Application EP 4 144 843 A1, published March 8, 2023. Title: IMMUNE CELL TREATED BY MEANS OF MAGNETIC FIELD AND USE THEREOF. Applicant: HEYE HEALTH TECHNOLOGY CO., LTD. CENTER FOR EXCELLENCE IN MOLECULAR CELL SCIENCE, CHINESE ACADEMY OF SCIENCES. The sequence listing filed with the application follows.

SEQUENCE LISTING (51 sequences)

SEQ ID NO: 1 - DNA, 22 bp, Artificial Sequence
  primer
gacggccaggtcatcactattg

SEQ ID NO: 2 - DNA, 20 bp, Artificial Sequence
  primer
aggaaggctggaaaagagcc

SEQ ID NO: 3 - DNA, 20 bp, Artificial Sequence
  primer
cacggtcgaagttctatgtc

SEQ ID NO: 4 - DNA, 24 bp, Artificial Sequence
  primer
ttgtgtgtttggatgagataaatc

SEQ ID NO: 5 - DNA, 21 bp, Artificial Sequence
  primer
agttgctctacctcgggatct

SEQ ID NO: 6 - DNA, 21 bp, Artificial Sequence
  primer
atgccacatcaaagcgaaagc

SEQ ID NO: 7 - DNA, 20 bp, Artificial Sequence
  primer
aggcacaagatgtgagggtg

SEQ ID NO: 8 - DNA, 20 bp, Artificial Sequence
  primer
cagcagccttgaacacttcc

SEQ ID NO: 9 - DNA, 21 bp, Artificial Sequence
  primer
ggggaaaagatcacgcatacc

SEQ ID NO: 10 - DNA, 22 bp, Artificial Sequence
  primer
caaaacgaaccctcctgtagtc

SEQ ID NO: 11 - DNA, 20 bp, Artificial Sequence
  primer
gagttcacctatgactacca

SEQ ID NO: 12 - DNA, 22 bp, Artificial Sequence
  primer
ctagaataatggagatgcgaat

SEQ ID NO: 13 - DNA, 21 bp, Artificial Sequence
  primer
aaagttgccccgaaggttaaa

SEQ ID NO: 14 - DNA, 23 bp, Artificial Sequence
  primer
gagcatagttttccagagaagca

SEQ ID NO: 15 - DNA, 19 bp, Artificial Sequence
  primer
ggccgatctgctgtttcag

SEQ ID NO: 16 - DNA, 21 bp, Artificial Sequence
  primer
catctcgcattaaccccagtt

SEQ ID NO: 17 - DNA, 19 bp, Artificial Sequence
  primer
acggccccatcgactacaa

SEQ ID NO: 18 - DNA, 22 bp, Artificial Sequence
  primer
cctggttccacctcatcattct

SEQ ID NO: 19 - DNA, 22 bp, Artificial Sequence
  primer
gttcaggtctctccactcatca

SEQ ID NO: 20 - DNA, 22 bp, Artificial Sequence
  primer
cggggttttaggtaactgtagc

SEQ ID NO: 21 - DNA, 21 bp, Artificial Sequence
  primer
gagccacctgttctggatgtg

SEQ ID NO: 22 - DNA, 23 bp, Artificial Sequence
  primer
gcacgacgatagtcagagaagtc

SEQ ID NO: 23 - DNA, 20 bp, Artificial Sequence
  primer
ttgcccttagccaaaaacgc

SEQ ID NO: 24 - DNA, 21 bp, Artificial Sequence
  primer
tcatggaaactaggtgccctc

SEQ ID NO: 25 - DNA, 21 bp, Artificial Sequence
  primer
acctttcactacctgcggatg

SEQ ID NO: 26 - DNA, 20 bp, Artificial Sequence
  primer
gtacccaggggcatacttgc

SEQ ID NO: 27 - DNA, 20 bp, Artificial Sequence
  primer
ccaacaacaacgacaatcta

SEQ ID NO: 28 - DNA, 20 bp, Artificial Sequence
  primer
ttgagtgtagtagtgctgaa

SEQ ID NO: 29 - DNA, 21 bp, Artificial Sequence
  primer
ctcttctacttccactaccat

SEQ ID NO: 30 - DNA, 23 bp, Artificial Sequence
  primer
gcctagagatagaattgtgacta

SEQ ID NO: 31 - DNA, 20 bp, Artificial Sequence
  primer
cttcttcaacctcaccatag

SEQ ID NO: 32 - DNA, 20 bp, Artificial Sequence
  primer
cttccaggcatagtaatgtg

SEQ ID NO: 33 - DNA, 22 bp, Artificial Sequence
  primer
ggtaatgaatgaggcaaataga

SEQ ID NO: 34 - DNA, 23 bp, Artificial Sequence
  primer
gtaatgaatgaggcaaatagatt

SEQ ID NO: 35 - DNA, 21 bp, Artificial Sequence
  primer
tctcgaccctacatggcctta

SEQ ID NO: 36 - DNA, 22 bp, Artificial Sequence
  primer
tcctgttctttgatgttgtggg

SEQ ID NO: 37 - DNA, 23 bp, Artificial Sequence
  primer
ctggatgtcaatcaacaatggga

SEQ ID NO: 38 - DNA, 23 bp, Artificial Sequence
  primer
actagggtgtgagtgttttctgt

SEQ ID NO: 39 - DNA, 20 bp, Artificial Sequence
  primer
tcctcgccagactcgttttc

SEQ ID NO: 40 - DNA, 21 bp, Artificial Sequence
  primer
gtcttgggtcattgctggaag

SEQ ID NO: 41 - DNA, 21 bp, Artificial Sequence
  primer
cttaaagacaaacctgagcat

SEQ ID NO: 42 - DNA, 20 bp, Artificial Sequence
  primer
ttccacatagtccatctctg

SEQ ID NO: 43 - DNA, 21 bp, Artificial Sequence
  primer
ttgaagagttactgcttgatg

SEQ ID NO: 44 - DNA, 21 bp, Artificial Sequence
  primer
acgcctaatatagtctccatt

SEQ ID NO: 45 - DNA, 19 bp, Artificial Sequence
  primer
tgtgggcatcaaccgatgg

SEQ ID NO: 46 - DNA, 21 bp, Artificial Sequence
  primer
cggactacaaacagacgcgaa

SEQ ID NO: 47 - DNA, 97 bp, Artificial Sequence
  shRNA primer
tgctgttgacagtgagcgcaagaagtgatcttttagttaatagtgaagccacagatgtattaactaaaagatcacttcttttgcctactgcctcgga

SEQ ID NO: 48 - DNA, 97 bp, Artificial Sequence
  shRNA primer
tgctgttgacagtgagcgcgccattgatttgatagcacaatagtgaagccacagatgtattgtgctatcaaatcaatggcatgcctactgcctcgga

SEQ ID NO: 49 - DNA, 97 bp, Artificial Sequence
  shRNA primer
tgctgttgacagtgagcgatgcctcgtgggtgaaaataaatagtgaagccacagatgtatttattttcacccacgaggcagtgcctactgcctcgga

SEQ ID NO: 50 - DNA, 97 bp, Artificial Sequence
  shRNA primer
tgctgttgacagtgagcgcccgcctctttatttacatctatagtgaagccacagatgtatagatgtaaataaagaggcggatgcctactgcctcgga

SEQ ID NO: 51 - DNA, 97 bp, Artificial Sequence
  shRNA primer
tgctgttgacagtgagcgccagtttgtttgtgaatatttatagtgaagccacagatgtataaatattcacaaacaaactgttgcctactgcctcgga